European Patent Specification EP 3 938 542 B1, published August 27, 2025. Title: IMPROVED METHOD FOR THE SCREENING, DIAGNOSIS AND/OR MONITORING OF COLORECTAL ADVANCED NEOPLASIA, ADVANCED ADENOMA AND/OR COLORECTAL CANCER. Applicant: GOODGUT S.L. Fundacio Institut d'Investigació Biomèdica de Girona Dr. Josep Trueta Universitat de Girona. The sequence listing filed with the application follows.

SEQUENCE LISTING (33 sequences)

SEQ ID NO: 1 - DNA, 783 bp, Gemella morbillorum
  misc_feature (1)..(783): GenBank access number: LS483440.1 REGION: 827110..827892
atggcgagtttattacaaaaaacaagaaaaataagtacaattttacaagaaggacgtcatgataatgtcgattttgaagcaatggcaatgcgcttaagtcctattttagattctgttgtctatattttagatgtagaaggtaatattcttgggtatgattctattgtagattattctaacgaacgtatggaagaaattattcgtgcgaggaaagtgcctaaagcttatttagatgcaacattaaaagtatatgctacgaaggttaatattccatttcaagatccgctttctattttcccagatgaagagaaagaaagatttgatgggaatacctatactgtaattttaccaataagaggcgggggagaacgccttggaactcttgttataggaagaatggataatgactttcaagatgatgatttggtgttagcagaatatgcgtcaacagtagtaggaattgaaattcttcacgaaaaacaagataaagaaaaaaatctagctagagacaaagatatggtgaatatggctcttaattcgttatcatattcagaaaaagaagcaattgaacatattttcagagaattagatgggacagaaggactacttatcgcaagtaaaattgcagatagagtaggaattactcgctcagttattgttaatgcacttagaaaattagaaagtgcaggtattatagagtcaaaatcattaggtatgaaaggtacttatataaaagtacttaaagaatattttttagaattaatgttttctaatgaattttaa

SEQ ID NO: 2 - DNA, 567 bp, Peptostreptococcus stomatis DSM 17678 strain
  misc_feature (1)..(567): GenBank access number: ADGQ01000060.1 REGION: complement (142796..143362)
atggatattattcaacttagcaacagacttatagaatacagaaaaagtaacaacttaactattaaagatttctctgacatgtccggaattagtactgctctgcttagtcaattagaaagaggtgttggaaaccctagcctgagtgtattgaactctatagcagataccatgaatactagcctctcctctttattagaagaacctgttgttttagaaaacctggttagaaggtctgacaccctatccactattgtctacccatgtaggaacaaccttgaatttcagttgctcacaactaggtctactactcagagcatcaaccttgtaagaataatatttcatgctcattcagaaactaattaccagccacttggaaaaaccgtttctgatgatataatccacattgaaaagggcagtattattgttcaaactgatgatggtaagtctattcaactaaaaaaaggtgatactatgaggataccacctgaccttaggtataaattcaagaatatttctgtacacaaggcacatatgatttgtgccactaataaacttgaagtaagataa

SEQ ID NO: 3 - DNA, 717 bp, Bacteroides fragilis
  misc_feature (1)..(717): GenBank access number: CR626927.1 REGION: 417101..417817
atggcaaatactaatatggaacacggagaaataatactataccaaccagacaatactataaaactggaagtgcgaatagagaatgaaaccgtttggttgacacaagcacaaattgttaacttattccagtcaagtaaagccaatatcagtgagcatataagaaatatatatgactcagatgaattatctgctgaatcaactgttcggaaattccgaacagttcgaatggaaggtaatagaaaggttacccgcattcttgaatattataatctggatatgattatttccgtaggttatcgtgtgaattccaagcgaggagtccagttccgccaatggtcaacaggagtacttaaagaatatctattaaaaggctacgcaatcaatcagcgcgtggagcagttggaaaacaaagcaaacacccatgaccggcaactggaagagttaacaaacaaagtcgactttttcgtccggacttcattacctcctattgaaggtgtctttttcaacggacagattttcgatgcctatgtcttttccgctcagttgataaagtctgcaaagtcatctttagtattgattgacaactttgtcgatgaaagcgtgctcttactattgagtaaacgtttgcccggagtgacttctatcatatataccaagcaagtaactccacagttagaattagatttgacaaagcacaacagtcaatacccccaatag

SEQ ID NO: 4 - DNA, 642 bp, Bacteroides thetaiotaomicron
  misc_feature (1)..(642): GenBank access number: AE015928.1 REGION: 326008..326649
atggcagtacaatttgaattatataagactccgatgccaaaggagaaaaagaacaagacgcgttatcatgcccgtccggtaagttttgagaccgtcaataccgagaaactggcttatcgcatccatgatcgctccacattaagagtatcggacattatttcaaccttggaagaactgaaaaatgaagtagctcagtgcctcctggaaggtaaaaaggtgcatgtcgatggattaggattctttcaggtcactctttcctgcgaagaagaaatacgtaacccgaaagacaaacgtgtgcaccgggtaaaattgaaagctataaagtttaaagctgataaagaattgaaaggggaattgtgtcacatgaaattccagcgttctaaaatcagaccgcactccgccaatttatcagaagtagaaatagacatgaaactaactgaatattttgctgaaaatcagattatcacccggaaagattttcaatatctctgcggaatgacacaaatcactgcatatcgccatatcaagaggttaatggcagaaaagaaattgcaaaataaagggacgatctatcaaccgatatatactccggttccgggtaattacagggtatcggtggatttaaaatataaagaacaatga

SEQ ID NO: 5 - DNA, 21 bp, Artificial Sequence
  EUB2 forward primer
  misc_feature (1)..(21)
actcctacgggaggcagcagt

SEQ ID NO: 6 - DNA, 22 bp, Artificial Sequence
  EUB2 reverse primer
  misc_feature (1)..(22)
gtattaccgcggctgctggcac

SEQ ID NO: 7 - DNA, 485 bp, Artificial Sequence
  B10; uncultured bacterium isolate DGGE gel band Eub_10 16S ribosomal RNA gene
  misc_feature (1)..(485)
cttcggattgtaaactcctgttgttgaggagataatgacggtactcaacaaggtaagtgacggctaactacgtgccagcagccgcggtaaaacgtaggtcacaagcgttgtccggaattactgggtgtaaagggagcgcaggcgggaagacaagttggaagtgaaatccatgggctcaacccatgaactgctttcaaaactgtttttcttgagtagtgcacaggtaggcggaattcccggtgtagcggtggaatgcgtagatatcgggaggaacaccagtggcgaaggcggcctactgggcaccaactgacgctgaggctcgaaagtgtgggtagcaaacaggattagataccctggtagtccacactgtaaacgatgattactaggtgttggaggattgaccccttcagtgccgcagttaacacaataagtaatccacctggggagtacgaccgcaaggttgaaactcaaaggaattgacggac

SEQ ID NO: 8 - DNA, 474 bp, Artificial Sequence
  B46; uncultured bacterium isolate DGGE gel band Eub_46 16S ribosomal RNA gene
  misc_feature (1)..(474)
gtaacatttctgtaacaagacatacagcagtttctcagagttcccaaactcaaaggaattgacggaagccgcggttccacgtaagtcacaagcgttgtccggaattactgggtgtaaagggagcgcaggcgggaagacaagttggaagtgaaatccatgggctcaacccataaactgctttcctaactgtttttcttgagtagtgcacaggtaggcggaattcccggtgtagcggtggaatgcctagatatcgggaggaacaccattggcgaaggcggcctactggactgcaactgacgctgaggctcgaaagtgtgggtagcaaacaggattagataccctggtagtccactccgtaaaccatgattactacgtgttggaggattgaccccttctgtgccgcagataacacaataagtaatccacctggggagtacgaccgcccggttgagactcacaggaattgacggactc

SEQ ID NO: 9 - DNA, 566 bp, Artificial Sequence
  B48; uncultured bacterium isolate DGGE gel band Eub_48 16S ribosomal RNA gene
tctcttacggggagcagcagtggggaatattgcacaatgggggaaaccctgatgcagcgacgccgcgtgagcgatgaagtatttcggtatgtaaagctctatcagcagggaagaaaatgacggtacctgactaagaagccccggctaaatacgtgccagcagccgcggtaatacgtatggtgcaagcgttatccggatttactgggtgtaaagggagcgtagacggagtggcaagtctgatgtgaaaacccggggctcaaccccgggactgcattggaaactgtgcatctagagtgtcggagaggtaagcggaattcctagtgtagcggtgaaatgcgtagatattaggaggaacaccagtggcgaaggcggcttactggacgataactgacgctgaggctcgaaagcgtggggagcaaacaggattagataccctggtagtccacgccgtaaacgatgactactaggtgtcggggagcacagctcttcggtgccgcagcaaacgcaataagtattccacctggggagtacgttcgcaagaatgaaactcacagaatttgacggag

SEQ ID NO: 10 - DNA, 894 bp, Rosburia intestinalis L1-82 strain
  misc_feature (1)..(894): GenBank access number LR027880.1 REGION: 599208..600101
atgtctttttcaagtgaagtgaaacaggagttagcaaagcagagtggaaagagcagacattgtcagatcgctgaacttgcggcgttagttgcttttgacggaaagcgtcagcagctgatcggggatgcgggagatgtgctggattcggaaaatccgcttctgcaggaaaaatatggactgttactggcacagctgttccatgttaatatagaagagatagatacattgccaccggaacgcattcttgagacaatcaagatgtggaatcagtctttaaggtgtgcagatatcacagagacggtaaatggtattttactgcagcagacatgttgcaggcgggcatatatccggggagcatttttagcaggtggatcgatcagtgatccgaataagtcttatcattttgagattgtctgccgggaaattgcgcaggcgaaacagcttcaggatgcaatcaacagttttgagatggaagcaaagatcgtagaacgaaagaaacaccaggtcgtatatttaaaggaaggtgcccagatcgtggatatgttaaatatcatggaagcacatgtggcactgatgaatcttgaaaatgtgcgtatcttaaaagaaatgagaaattctgtcaaccgaaaggtaaattgtgagacggcaaatatcagcaagactgtggcggcagccgtaaaacagcttggcgatattgaatatattaaacagaatgcaggcttagacagtctgcctgaaaacctaaaagaaatggcgttgctgcggttagagtatccggatacaccgcttaaggaactgggaacatatctcgatcctccggtcggaaaatcgggagtgaaccacaggctgcgcaggatcagtgagattgcagatgagctgcgtgaaaaagaataa

SEQ ID NO: 11 - DNA, 807 bp, Collinsella intestinalis DSM 13280 strain
  misc_feature (1)..(807): NCBI Reference Sequence: GG692711.1 REGION: 297314..298120
atgtccggacactctaaatgggcaactaccaagcaccgcaagggtgcgcaggacgctaagcgttccgccctgttctccaagctgagccgtaacatcaccgtcgcggcccgtcttggcaacgaccccaacccggacaacaacgcctccctcgccgctgccgtggccaaggccaaggctcagtccatgcccaaggacaagatcaaggccgccatcgacaaggccttcggttccggcgccgacgccgccgtgtacgagaacatcgtgtacgagggctacggcccggccggtgttgccgtgtacgtcgagtgcctgaccgacaaccgcaaccgcaccgccgccgatgtccgctccgccttctcccacgctggcggcaacctgggcaccaccggctccgttgccttccagttcgagcgcaagggccaggtcgtggtctccaagcagatcgtcgacccgaacgacaagaaggagaacctcatggccaacggcgctgccggcgatgaggaagagttcatgatggtcatcgccgaggccggtggcgacgactacgaggacgccggtgacgagtgggtcgtgtggaccgccgcgggcgacctcatggccgtgtccaagggcatcgaggctcagggcatcgaggtcaagggtgccgagctcaccatggtcccgaccaccccgacggccgtctccggcgccgacgccaagaaggtccagcgcctcatcgaccgcctcgaggacctggacgacgtccaggacgtgtactccaccatggacatgaccgacgaggtcatcgctgccctcgaagaggagtaa

SEQ ID NO: 12 - DNA, 1466 bp, Faecalibacterium prausnitzii
  misc_feature (1)..(1466): GenBank access number: AJ270469.2
gttgatcctggctcaggacgaacgctggcggcgcgcctaacacatgcaagtcgaacgagcgagagagagcttgctttctcgagcgagtggcgaacgggtgagtaacgcgtgaggaacctgcctcaaagagggggacaacagttggaaacgactgctaataccgcataagcccacagctcggcatcgagcagagggaaaaggagcaatccgctttgagatggcctcgcgtccgattagctagttggtgaggtaatggcccaccaaggcaacgatcggtagccggactgagaggttgaacggccacattgggactgagacacggcccagactcctacgggaggcagcagtggggaatattgcacaatgggggaaaccctgatgcagcgacgccgcgtggaggaagaaggtcttcggattgtaaactcctgttgttgaggaagataatgacggtactcaacaaggaagtgacggctaactacgtgccagcagccgcggtaaaacgtaggtcacaagcgttgtccggaattactgggtgtaaagggagcgcaggcgggaagacaagttggaagtgaaatctatgggctcaacccataaactgctttcaaaactgtttttcttgagtagtgcagaggtaggcggaattcccggtgtagcggtggaatgcgtagatatcgggaggaacaccagtggcgaaggcggcctactgggcaccaactgacgctgaggctcgaaagtgtgggtagcaaacaggattagataccctggtagtccacaccgtaaacgatgattactaggtgttggaggattgaccccttcagtgccgcagttaacacaataagtaatccacctggggagtacgaccgcaaggttgaaactcaaaggaattgacgggggcccgcacaagcagtggagtatgtggtttaattcgacgcaacgcgaagaaccttaccaagtcttgacatcctgcgacgatgctggaaacagtattttccttcgggacgcagagacaggtggtgcatggttgtcgtcagctcgtgtcgtgagatgttgggttaagtcccgcaacgagcgcaacccttactgtcagttactacgcaagaggactctggcaggactgccgttgacaaaacggaggaaggtggggatgacgtcaaatcatcatgccctttatgacttgggctacacacgtactacaatggcgttaaacaaagagaagcaagaccgcgaggtggagcaaaactcagaaacaacgtcccagttcggactgcaggctgcaactcgcctgcacgaagtcggaattgctagtaatcgtggatcagcatgccacggtgaatacgttcccgggccttgtacacaccgcccgtcacaccatgagagccggggggacccgaagtcggtagtctaaccgcaaggaggacgccgccgaaggtaaaactggtgattggggtgaagtcgtaacaaggtac

SEQ ID NO: 13 - DNA, 1452 bp, Escherichia coli
  misc_feature (1)..(1452)
cgccctcccgaaggttaagctacctacttcttttgcaacccactcccatggtgtgacgggcggtgtgtacaaggcccgggaacgtattcaccgtggcattctgatccacgattactagcgattccgacttcatggagtcgagttgcagactccaatccggactacgacgcactttatgaggtccgcttgctctcgcgaggtcgcttctctttgtatgcgccattgtagcacgtgtgtagccctggtcgtaagggccatgatgacttgacgtcatccccaccttcctccagtttatcactggcagtctcctttgagttcccggccggaccgctggcaacaaaggataagggttgcgctcgttgcgggacttaacccaacatttcacaacacgagctgacgacagccatgcagcacctgtctcacggttcccgaaggcacattctcatctctgaaaacttccgtggatgtcaagaccaggtaaggttcttcgcgttgcatcgaattaaaccacatgctccaccgcttgtgcgggcccccgtcaattcatttgagttttaaccttgcggccgtactccccaggcggtcgacttaacgcgttagctccggaagccacgcctcaagggcacaacctccaagtcgacatcgtttacggcgtggactaccagggtatctaatcctgtttgctccccacgctttcgcacctgagcgtcagtcttcgtccagggggccgccttcgccaccggtattcctccagatctctacgcatttcaccgctacacctggaattctacccccctctacgagactcaagcttgccagtatcagatgcagttcccaggttgagcccggggatttcacatctgacttaacaaaccgcctgcgtgcgctttacgcccagtaattccgattaacgcttgcaccctccgtattaccgcggctgctggcacggagttagccggtgcttcttctgcgggtaacgtcaatgagcaaaggtattaactttactcccttcctccccgctgaaagtactttacaacccgaaggccttcttcatacacgcggcatggctgcatcaggcttgcgcccattgtgcaatattccccactgctgcctcccgtaggagtctggaccgtgtctcagttccagtgtggctggtcatcctctcagaccagctagggatcgtcgcctaggtgagccgttaccccacctactagctaatcccatctgggcacatccgatggcaagaggcccgaaggtccccctctttggtcttgcgacgttatgcggtattagctaccgtttccagtagttatccccctccatcaggcagtttcccagacattactcacccgtccgccactcgtcagcaaagaagcaagcttcttcctgttaccgttcgacttgcatgtgttaggcctgccgccagcgttcaatctgagccatgatcaaact

SEQ ID NO: 14 - DNA, 21 bp, Artificial Sequence
  EUB_F forward primer
  misc_feature (1)..(21)
actcctacgggaggcagcagt

SEQ ID NO: 15 - DNA, 22 bp, Artificial Sequence
  EUB_R reverse primer
  misc_feature (1)..(22)
gtattaccgcggctgctggcac

SEQ ID NO: 16 - DNA, 19 bp, Artificial Sequence
  B10_F primer forward
  misc_feature (1)..(19)
caacaaggtaagtgacggc

SEQ ID NO: 17 - DNA, 20 bp, Artificial Sequence
  B10_R reverse primer
  misc_feature (1)..(20)
cgcctacctgtgcactactc

SEQ ID NO: 18 - DNA, 19 bp, Artificial Sequence
  B46_F forward primer
  misc_feature (1)..(19)
tccacgtaagtcacaagcg

SEQ ID NO: 19 - DNA, 20 bp, Artificial Sequence
  B46_R reverse primer
  misc_feature (1)..(20)
cgcctacctgtgcactactc

SEQ ID NO: 20 - DNA, 18 bp, Artificial Sequence
  B48_F forward primer
gtacggggagcagcagtg

SEQ ID NO: 21 - DNA, 23 bp, Artificial Sequence
  B48_R reverse primer
  misc_feature (1)..(23)
gacactctagatgcacagtttcc

SEQ ID NO: 22 - DNA, 20 bp, Artificial Sequence
  GMLL_F forward primer
aagagttccaaggcgttctc

SEQ ID NO: 23 - DNA, 25 bp, Artificial Sequence
  GMLL_R reverse primer
  misc_feature (1)..(25)
ccatttcaagatccgctttctattt

SEQ ID NO: 24 - DNA, 22 bp, Artificial Sequence
  PTST_F forward primer
  misc_feature (1)..(22)
aggttgatgctctgagtagtag

SEQ ID NO: 25 - DNA, 23 bp, Artificial Sequence
  PTST_R reverse primer
  misc_feature (1)..(23)
atgaatactagcctctcctcttt

SEQ ID NO: 26 - DNA, 22 bp, Artificial Sequence
  BCTF_F forward primer
  misc_feature (1)..(22)
tgaaagcgtgctcttactattg

SEQ ID NO: 27 - DNA, 20 bp, Artificial Sequence
  BCFT_R reverse primer
  misc_feature (1)..(20)
tattggctgttgtgctttgt

SEQ ID NO: 28 - DNA, 21 bp, Artificial Sequence
  CINT_F forward primer
  misc_feature (1)..(21)
gaccatcatgaactcttcctc

SEQ ID NO: 29 - DNA, 17 bp, Artificial Sequence
  CINT_R reverse primer
  misc_feature (1)..(17)
ccgttgccttccagttc

SEQ ID NO: 30 - DNA, 22 bp, Artificial Sequence
  BCTT_F forward primer
  misc_feature (1)..(22)
agtgacctgaaagaatcctaat

SEQ ID NO: 31 - DNA, 20 bp, Artificial Sequence
  BCTT_R reverse primer
  misc_feature (1)..(20)
gaccgtcaataccgagaaac

SEQ ID NO: 32 - DNA, 21 bp, Artificial Sequence
  RSBI_F forward primer
  misc_feature (1)..(21)
gtgccagtaacagtccatatt

SEQ ID NO: 33 - DNA, 20 bp, Artificial Sequence
  RSBI_R reverse primer
  misc_feature (1)..(20)
tagcaaagcagagtggaaag